European Patent Specification EP 3 733 865 B1, published October 15, 2025. Title: Method for obtaining single-cell mRNA sequence. Applicant: MGI TECH CO., LTD. The sequence listing filed with the application follows.

SEQUENCE LISTING (28 sequences)

SEQ ID NO: 1 - DNA, 35 bp, Artificial sequence
cttccggcagaacgacatggctacgaaaaaaaaaa

SEQ ID NO: 2 - DNA, 20 bp, Artificial sequence
cgtagccatgtcgttctgcc

SEQ ID NO: 3 - DNA, 26 bp, Artificial sequence
  misc_feature (1)..(10): n is a, c, g, or t
nnnnnnnnnnaccctgactaggtcgc

SEQ ID NO: 4 - DNA, 37 bp, Artificial sequence
  misc_feature (22)..(31): n is a, c, g, or t
ggaaggcgacctagtcagggtnnnnnnnnnncgcaga

SEQ ID NO: 5 - DNA, 69 bp, Artificial sequence
  misc_feature (54)..(63): n is a, c, g, or t
gcactgacgacatgatcaccaaggatcgatagtccatgctaggcgtcgttttannnnnnnnnntctgcg

SEQ ID NO: 6 - DNA, 20 bp, Artificial sequence
  misc_feature (1)..(10): n is a, c, g, or t
nnnnnnnnnntaaaacgacg

SEQ ID NO: 7 - DNA, 27 bp, Artificial sequence
tttttcccgtagccatgtcgttctgcg

SEQ ID NO: 8 - DNA, 16 bp, Artificial sequence
acgacatggctacggg

SEQ ID NO: 9 - DNA, 22 bp, Artificial sequence
  misc_feature (1)..(10): n is a, c, g, or t
nnnnnnnnnnacctgagatcgc

SEQ ID NO: 10 - DNA, 34 bp, Artificial sequence
  misc_feature (19)..(28): n is a, c, g, or t
ggaagggcgatctcaggtnnnnnnnnnncgcaga

SEQ ID NO: 11 - DNA, 53 bp, Artificial sequence
  misc_feature (7)..(16): n is a, c, g, or t
  misc_feature (22)..(31): n is a, c, g, or t
ccttccnnnnnnnnnncgatgnnnnnnnnnntttttttttttttttttttttv

SEQ ID NO: 12 - DNA, 15 bp, Artificial sequence
  misc_feature (6)..(15): n is a, c, g, or t
catcgnnnnnnnnnn

SEQ ID NO: 13 - DNA, 23 bp, Artificial sequence
cgtagccatgtcgttctgrgrgg

SEQ ID NO: 14 - DNA, 18 bp, Artificial sequence
cgtagccatgtcgttctg

SEQ ID NO: 15 - DNA, 73 bp, Artificial sequence
cctagcatggactatcgatccttggtgatcatgtcgtcagtgcttgtcttcctaagatgtgtataagagacag

SEQ ID NO: 16 - DNA, 19 bp, Artificial sequence
ctgtctcttatacacatct

SEQ ID NO: 17 - DNA, 41 bp, Artificial sequence
gagacgttctcgactcagcagaagatgtgtataagagacag

SEQ ID NO: 18 - DNA, 19 bp, Artificial sequence
ctgtctcttatacacatct

SEQ ID NO: 19 - DNA, 43 bp, Artificial sequence
cctagcatggactatcgatccttggtgatcatgtcgtcagtgc

SEQ ID NO: 20 - DNA, 42 bp, Artificial sequence
cgtagccatgtcgttctgccggaagggcgacctagtcagggt

SEQ ID NO: 21 - DNA, 18 bp, Artificial sequence
cgtagccatgtcgttctg

SEQ ID NO: 22 - DNA, 22 bp, Artificial sequence
gagacgttctcgactcagcaga

SEQ ID NO: 23 - DNA, 26 bp, Artificial sequence
aagcduducgtagccatgtcgttctg

SEQ ID NO: 24 - DNA, 16 bp, Artificial sequence
tttttttttttttttt

SEQ ID NO: 25 - DNA, 42 bp, Artificial sequence
ggaaacagctatgaccatgcgtagccatgtcgttctgrgrgg

SEQ ID NO: 26 - DNA, 18 bp, Artificial sequence
cgtagccatgtcgttctg

SEQ ID NO: 27 - DNA, 19 bp, Artificial sequence
ggaaacagctatgaccatg

SEQ ID NO: 28 - DNA, 24 bp, Artificial sequence
gacatggctacgggaaacagctat